European Patent Application EP 4 285 728 A1, published December 6, 2023. Title: Composition comprising non-starch polysaccharide degrading enzymes. Applicant: Kerry Group Services International Limited. The sequence listing filed with the application follows.

SEQUENCE LISTING (49 sequences)

SEQ ID NO: 1 - protein, 223 aa, Unknown
  Unknown
MVSFTSLLAGVAAISGVLAAPAAEVESVAVEKRQTIQPGTGYNNGYFYSYWNDGHGGVTYTNGPGGQFSVNWSNSGNFVGGKGWQPGTKNKVINFSGSYNPNGNSYLSVYGWSRNPLIEYYIVENFGTYNPSTGATKLGEVTSDGSVYDIYRTQRVNQPSIIGTATFYQYWSVRRNHRSSGSVNTANHFNAWAQQGLTLGTMDYQIVAVEGYFSSGSASITVS

SEQ ID NO: 2 - protein, 347 aa, Unknown
  Unknown
MKANVILCLLAPLVAALPTETIHLDPELAALRANLTERTADLWDRQASQSIDQLIKRKGKLYFGTATDRGLLQREKNAAIIQADLGQVTPENSMKWQSLENNQGQLNWGDADYLVNFAQQNGKSIRGHTLIWHSQLPAWVNNINNADTLRQVIRTHVSTVVGRYKGKIRAWDVVNEIFNEDGTLRSSVFSRLLGEEFVSIAFRAARDADPSARLYINDYNLDRANYGKVNGLKTYVSKWISQGVPIDGIGSQSHLSGGGGSGTLGALQQLATVPVTELAITELDIQGAPTTDYTQVVQACLSVSKCVGITVWGISDKDSWRASTNPLLFDANFNPKPAYNSIVGILQ

SEQ ID NO: 3 - protein, 229 aa, Unknown
  Unknown
MVAFSSLICALTSIASTLAMPTGLEPESSVNVTERGMYDFVLGAHNDHRRRASINYDQNYQTGGQVSYSPSNTGFSVNWNTQDDFVVGVGWTTGSSAPINFGGSFSVNSGTGLLSVYGWSTNPLVEYYIMEDNHNYPAQGTVKGTVTSDGATYTIWENTRVNEPSIQGTATFNQYISVRNSPRTSGTVTVQNHFNAWASLGLHLGQMNYQVVAVEGWGGSGSASQSVSN

SEQ ID NO: 4 - protein, 152 aa, Unknown
  Unknown
MGPLEESINANITERGPNNFVLGGHNAVRRAAINYNQDYTTGGDVVYTHSNTGFAVNWSYPNDFVVGVGWNPGGSAPINFSGNFGVGSGVGLLSVYGWSTNPLVEYYVVEDNFGFSSGGTVKGSVTSDGSSYTIWENTRVNEPSIVGTATFN

SEQ ID NO: 5 - protein, 426 aa, Unknown
  Unknown
MWVVYPPLKNFTGSNNYPDGIGQMQHFVNDDGMTIFRLPVGWQYLVNNNLGGNLDSTSISKYDQLVQGCLSLGAYCIVDIHNYARWNGGIIGQGGPTNAQFTSLWSQLASKYASQSRVWFGIMNEPHDVNINTWAATVQEVVTAIRNAGATSQFISLPGNDWQSAGAFISDGSAAALSQVTNPDGSTTNLIFDVHKYLDSDNSGTHAECTTNNIDGAFSPLATWLRQNNRQAILTETGGGNVQSCIQDMCQQIQYLNQNSDVYLGYVGWGAGSFDSTEASIPDLTGRVALVTGGNHIGHFVLTTKLLPLLKATASTTGSDVRIVTISSVAEKFAPRHNTFATTKDLSDPGTADPNDYTSRKTVFSRYGASKLANLLFTRELQRRLDEEDANIMALAVDPGPVATDGGMGVFPGFLKPVLKLVMKSP

SEQ ID NO: 6 - protein, 459 aa, Unknown
  Unknown
MAPSVTLPLTTAILAIARLVAAQQPGTSTPEVHPKLTTYKCTKSGGCVAQDTSVVLDWNYRWMHDANYNSCTVNGGVNTTLCPDEATCGKNCFIEGVDYAASGVTTSGSSLTMNQYMPSSSGGYSSVSPRLYLLDSDGEYVMLKLNGQELSFDVDLSALPCGENGSLYLSQMDENGGANQYNTAGANYGSGYCDAQCPVQTWRNGTLNTSHQGFCCNEMDILEGNSRANALTPHSCTATACDSAGCGFNPYGSGYKSYYGPGDTVDTSKTFTIITQFNTDNGSPSGNLVSITRKYQQNGVDIPSAQPGGDTISSCPSASAYGGLATMGKALSSGMVLVFSIWNDNSQYMNWLDSGNAGPCSSTEGNPSNILANNPNTHVVFSNIRWGDIGSTTNSTAPPPPPASSTTFSTTRRSSTTSSSPSCTQTHWGQCGGIGYSGCKTCTSGTTCQYSNDYYSQCL

SEQ ID NO: 7 - protein, 500 aa, Unknown
  Unknown
MVTGATGGLGSQLTRAILECGGDVIAIDAHEIPLATTWEPLKALAKSLSRTLVYHACDITSPSLLETVFESAASQVKHPLRGLVNCAGIGTAAESINYPESQTRQTLDVNLAGSLYVAQAAAKVVRRQYQEGKSPGASFVFVASMSGYIANKATPTAIYCASKAGVHQLTRSLAAEWGSPSSPLSAFSSSADAAAAAAATAAAGPVIRVNSISPGVIATPMTQQFLGRQDWTSTWQEEAMLKRISTPDEYRGAIAFLLGDASSYVTGTDLRIDGGSTGCFERYYDGQEGACGCGSSSGAFPWQLGIGNGVYTAAGSQALFDTAGASWCGAGCGKCYQLTSTGQAPCSSCGTGGAAGQSIIVMVTNLCPNNGNAQWCPVVGGTNQYGYSYHFDIMAQNEIFGDNVVVDFEPIACPGQAASDWGTCLCVGQQETDPTPVLGNDTGSTPPGSSPPATSSSPPSGGGQQTLYGQCGGAGWTGPTTCQAPGTCKVQNQWYSQCLP

SEQ ID NO: 8 - protein, 438 aa, Unknown
  Unknown
MRATSLLAAALAVAGDALAGKIKYLGVAIPGIDFGCDIDGSCPTDTSSVPLLSYKGGDGAGQMKHFAEDDGLNVFRISATWQFVLNNTVDGKLDELNWGSYNKVVNACLETGAYCMIDMHNFARYNGGIIGQGGVSDDIFVDLWVQIAKYYEDNDKIIFGLMNEPHDLDIEIWAQTCQKVVTAIRKAGATSQMILLPGTNFASVETYVSTGSAEALGKITNPDGSTDLLYFDVHKYLDINNSGSHAECTTDNVDAFNDFADWLRQNKRQAIISETGASMEPSCMTAFCAQNKAISENSDVYIGFVGWGAGSFDTSYILTLTPLGKPGNYTDNKLMNECILDQFTLDEKYRPTPTSISTAAEETATATATSDGDAPSTTKPIFREETASPTPNAVTKPSPDTSDSSDDDKDSAASMSAQGLTGTVLFTVAALGYMLVAF

SEQ ID NO: 9 - protein, 892 aa, Unknown
  Unknown
MMLSKSLLSAATAASALAAVLQPVPRASSFVTISGTQFNIDGKVGYFAGTNCYWCSFLTNHADVDSTFSHISSSGLKVVRVWGFNDVNTQPSPGQIWFQKLSATGSTINTGADGLQTLDYVVQSAEQHNLKLIIPFVNNWSDYGGINAYVNAFGGNATTWYTNTAAQTQYRKYVQAVVSRYANSTAIFAWELGNEPRCNGCSTDVIVQWATSVSQYVKSLDSNHLVTLGDEGLGLSTGDGAYPYTYGEGTDFAKNVQIKSLDFGTFHLYPDSWGTNYTWGNGWIQTHAAACLAAGKPCVFEEYGAQQNPCTNEAPWQTTSLTTRGMGGDMFWQWGDTFANGAQSNSDPYTVWYNSSNWQCLVKNHVDAINGGTTTPPPVSSTTTTSSRTSSTPPPPGGSCSPLYGQCGGSGYTDRKIKCDRALPACTNCRQRNVPCPGYSIRLSWPRPGDKRRAVELKSTAKQKKHMLASLYQHSLFLNVTSWDVNTFYQLSEARSDMEIPKISIPPALPSIPSMRVHESQSGLLQYFMDMGPQLLVMDSSGDLTDWILRLAFYDATPASNAVLHSLLALSSLNLGRNSVAMMYKIMALSYLQQSLQLGNIGHRTAQHLMTSMLLYLCETFHISNTTKDWAEYLCGAKQIVSTGVLAREVHIDVSLLFDWVSYHETFARFGLVYWKPAVALRGLRFCAMSPETAQVFAPRNDFVCDRDVLGYTSSIFSSLTPRIKDNSHLSHLETQELYALEAKLRGGLMDFNPLNTLPDEAPKERDRITELYRLAALIYLNRAALGYSGEELRHRNLVNRGLDILCGKLTSTPPWPVFMIACEARDDAQRMTALEILDRAGEEPRSFNMRLIRQLVEACWNQDDLHEDEPLDYHTKLRIAIRAAPYVPPFS

SEQ ID NO: 10 - protein, 256 aa, Unknown
  Unknown
MVSFLGQARLAVPILSAFAWMFAASSAIPPPPPGTLSPERLQWIREVIGNQTEGGSISDIAKRSTILHTSQDGVDSGGFYYSVYNDNGASVGYTEYPTTGQFELGWNTETEFLGGKGFKGGSTRSLTWDGYFTAEGDWTLAIYGWTLNPVTEWYIVESHGTGTPGNGNILGQVDSDGGVYDVYNLPYRNVPEIYGVTNFDQHWSVRRSHRSTGTVDVSTHFQRWKELGLNPGTPIFQMVTLEGFSGQGYLDFTVQA

SEQ ID NO: 11 - protein, 225 aa, Unknown
  Unknown
MLTKNLLLCFAAAKAVLAVPHDSVVERSDALHKLSERSTPSSTGENNGYYYSFWTDGGGDVTYTNGNAGSYSVEWSNVGNFVGGKGWNPGSAKDITYSGTFTPSGNGYLSVYGWTTDPLIEYYIVESYGDYNPGSGGTYKGTVTSDGSVYDIYTASRTNAPSIQGTATFTQYWSVRQNKRVGGTVTTSNHFNAWAKLGMNLGTHNYQILATEGYQSSGSSSITIQ

SEQ ID NO: 12 - protein, 231 aa, Unknown
  Unknown
MVAYSSLLLALSAASSAVALPNGKALLDMAKRSLTSSAEGESNGYFYSFWTNGEGDVTYTNGDGGEYTVEWTDCGNFVAGKGWNPGSAQAVTYSGSWETDANAYLSVYGWTTSPLVEFYIVDKYGDYDPSSGLTELGTVDSDDGTYKIYQTTREDADSIEGTATFKQYWSVRTEGRIGGTVTTQNHFDAWENLGLELGTFNYMIVATEGYESSGSATITVDASSDSTEESC

SEQ ID NO: 13 - protein, 211 aa, Unknown
  Unknown
MKVTAAFAGLLVTAFAAPVPEPVLVSRSAGINYVQNYNGNLGDFTYDESAGTFSMYWEDGVSSDFVVGLGWTTGSSNAITYSAEYSASGSSSYLAVYGWVNYPQAEYYIVEDYGDYNPCSSATSLGTVYSDGSTYQVCTDTRTNEPSITGTSTFTQYFSVRESTRTSGTVTVANHFNFWAQHGFGNSDFNYQVMAVEAWSGAGSASVTISS

SEQ ID NO: 14 - protein, 321 aa, Unknown
  Unknown
MVQIKAAALAMLFASHVLSEPIEPRQASVSIDTKFKAHGKKYLGNIGDQYTLTKNSKTPAIIKADFGALTPENSMKWDATEPSRGQFSFSGSDYLVNFAQSNNKLIRGHTLVWHSQLPSWVQAITDKNTLIEVMKNHITTVMQHYKGKIYAWDVVNEIFNEDGSLRDSVFYKVIGEDYVRIAFETARAADPNAKLYINDYNLDSASYPKLAGMVSHVKKWIEAGIPIDGIGSQTHLSAGGALNALAGAGTKEIAVTELDIAGASSTDYVEVVEACLDQPKCIGITVWGVADPDSWRSSSTPLLFDSNYNPKPAYTAIANAL

SEQ ID NO: 15 - protein, 521 aa, Unknown
  Unknown
MRISNLIVAASAATMVSALPSRQMKKRDSGFKWVGTSESGAEFGSALPGTLGTDYTWPETSKIQVLRNKGMNIFRIPFLMERLTPDGLTGSFASTYLSDLKSTVEFVTNSGAYAVLDPHNYGRFDGSIIESTSDFKTWWKNVATEFADNDKVIFDTNNEYHDMEQSLVLNLNQAAINGIRAAGATTQYIFVEGNAYTGAWDWTTYNDDLSGLTDSEDKIIYEMHQYLDSDSSGTSETCVSSTIGKERIEKATEWLKTNNKQGIIGEFAGGVNSVCEEAVEGMLAYMSENSDVWVGASWWSAGPWWGTYMYSLEPTDGTAYSTYLPILEKYFPSGDASSSSSASASVAAATSAVSTTTTAAFEQTTTPATQVEIASSSSSSSAVAASQTTLSKVKSKSKSPCKLSSATSSAVSSAAAVTTPAVAATTPAAAPTSSSVAFATTSVYVPTTTAAAPSQVSSSAAASSSGVVGVSDPQGPSATNSAGEVNQYYQCGGINWTGPTVCASPYTCKVQNDYYYQCVAE

SEQ ID NO: 16 - protein, 411 aa, Unknown
  Unknown
MKTLSLVAVLLVQAWTASSSPRAKRSSGFQWFGSNESGAEFGSGNIPGTLGTDYIWPDATAIETLHSAGMNIFRVPFLMERLVPNELTGAADATYMADLKATVQTITDLGAYAVVDPHNFGRYYGNIITSTSDFAAFWTTVASEFTDNDLVIFDTNNEFHDEDQTLVLNLNQAAITAIRATGATTQYIFVEGNSYTGAWTWTTTNTNLVNLTDPNDHLIYEMHQYLDSDGSGTSSTCVSSTIGAERIADATSWLRENGKQAVLGEFAGGANSVCEEAVTGMLDAMVDASDVWLGGMWWSAGPWWGDYIFSLEPDDGVAYEYYLSVLEGYTPGSSSSSGGTTTTAAASTSSTSAAGSATTSKVTTTTAAATATSTAVAAHYAQCGGQGWTGATTCADGYTCTVENAWYSQCL

SEQ ID NO: 17 - protein, 452 aa, Unknown
  Unknown
MHQRALLFSALLTAVRAQQAGTLTEEVHPSLTWQKCTSEGSCTEQSGSVVIDSNWRWTHSVDGSTNCYTGNTWDSTLCPDDETCATNCALDGADYESTYGITTDGDSLTLKFVTGSNVGSRVYLMDTSDEKYQTFDLLDAEFTFDVDVSNLPCGLNGALYFTAMDADGGTSRYPANKAGAKYGTGYCDSQCPRDLKFINGEANVDGWEPSSNNDNTGIGNHGSCCPEMDIWEANSISTALTPHPCDSSKQTMCEGNNCGGTYSDDRYGGTCDPDGCDFNPFRMGNETFYGDGKIVDTGSKMTVVTQFITDGSSSLSEIKRYYVQNGNVIANAESSISGVTGNSITTDFCTAQKKAFGDDDVFAAHNGLAGISDAMSSMVLILSLWDDYYASMEWLDSDYPENATATDPGVARGTCDSESGVPATVEGAHPDASVTFSNIKFGPINSTFSASA

SEQ ID NO: 18 - protein, 536 aa, Unknown
  Unknown
MSSIDANWRWVHSTSSSTNCYTGNEWDTSICTDDVTCAANCALDGATYEATYGVTTSGDELRLNFVTQGSSKNIGSRLYLMSDDSTYEMFKLLGQEFTFDVDVSNLPCGLNGALYFVAMDADGGTSKYSGNKAGAKYGTGYCDSQCPRDLKFINGEANCDGWEPSSNNANTGVGDHGSCCPEMDVWEANSISNAFTAHPCDSTSQTMCDGDTCGGTYSASGDRYSGTCDPDGCDYNPYRLGDTDFYGPGLTVDTNSPFTVVTQFITDDGTSSGTLTEIKRLYVQNGKVIANGASTYSSVNGSSITSDFCEAQKTLFGDENVFDTHGGLAGMGEAMANGMVLVLSLWDDYASNMLWLDSDYPVDSSASTPGVARGTCSTDSGVPATVEAESPNAYVTYSNIKFGPIGSTYSSGSSSGSGSSSSSSSTTTKATSTTLKTTTTTSSGSSSTSAAQAYGQCGGQGWTGPTTCVSGYTCTYQNAYYSQCLFQIYRAALLLSILATANSQQVGTYTTETHPSLTWQTCTSSGSCTTNNGAVV

SEQ ID NO: 19 - protein, 737 aa, Unknown
  Unknown
MPTSSLLWSVGSLALSSMILPAAASGYQLVETWKGEDFLTAFDFYTGADPTNGFVTYANQSYAESKGLVKVNSNGSFYMGVDHTTKLSTNGPGRESVRIGSNKYYDEGLFIIDLEHMPGSVCGTWPAFWSTGKDWPTDGEIDIIEGVNKNEANEIVLHTSGTCQVSSQKMTGTLSSTECGEDSGTTGCVVEGTQGSSGNPFNENGGGVYAMQWTDEFLKFWFFPRGSIPTSITKGDPDVAAFGTPMAHMQGSCSIAEHFKAQQFIFDTTFCGDWAGGVYSTSGCPVSDSSSSFKSCVAYVAENPAAFAESYWEINYIKIYQTGVAASASASASRVESAATVVETVSSVKEVTNSVVATTAAATTVATTADAETATTMTIAETTTAAAATESSVADENGSSASTSTHYVTMTTTICPIAESSSAAADLAGGSSEATEGSNSEGSSATATPDSVTGASAESNGSEGSSATESTPSTATGASAEANGNESSSTSEASSVASGTPSDISTTGASAEANGSEDSSASSEAKAVASATPSSVTGASAEANGNDSASSNAATTSNVSGASTQAGDDESTPASAVANAGSSATPASVSGASAEANGSEQSAAAAASSVSGASAVANGSEGSSSQSSGSQAGSDSYGSVPSSAAAYGRPAPSSSSHAFSTAPSSSGSIRQPTSAAAANNDAAATQGSSASGSKSGHFGSGSSSATTPSTPVFTGGANKLTLGASSVVGVLAFALLA

SEQ ID NO: 20 - protein, 433 aa, Unknown
  Unknown
MRRTATLLSALGLTAQLSSAAYTLQDEYSGDSFFDGFTFFTGADPTNGFVDYVDEATAQSNGYISTSGDAPVYMGVDHTNIAGSSGRQSVRISSDATYNHGLFILDLGHMPGGVCGTWPAFWLVGADWPNNGEIDIIEGVNQQSGNDMTLHTSDGCSVSSSADFTGSMTTDNCYVSAAGQSNNAGCGITDPDGTSYGTAFNANNGGVFATEWTSDAISIWFFERGSIPDDIDSGNPDPDSWGSPVARFQGDCDIDAHFDNLQIIFDTTFCGDWAGNVWGSGSCASVASSCSDYVANNPEAFAEAYWIINSLKVYQDDGVDDDTVAGVVDYGDDEDDEDDQDDDNDDDDSDDDDDSDDDDDDDSDSDDDSDDDDDDDDDDDDDDDDDSRPWRGGGRNHHGSKLNASTSTSSFPSPSFVRKARWERRNPMAGMIF

SEQ ID NO: 21 - protein, 453 aa, Unknown
  Unknown
MLSKMQLAQLAAFAMTLATSEAAYQGFNYGNKFSDESSKFQADFEAEFKAAKNLQTTSGFTSARLYTMIQAYSTSDVIEAIPAAIAQDTSLLLGLWASGGGMDNEITALKTAISQYGEELGKLVVGISVGSEDLYRNSVEGVEADAGVGVNPDELVSYIKEVRSVISGTALADVSIGHVDTWDSWTNSSNSAVVEAVDWLGFDGYPFFQSSMANSIDNAKSLFEESVEKTKAVAGDKEVWITETGWPVSGDSQGDAVASIANAKKFWDEVGCPLFGNVNTWWYILQDASPTTPNPSFGIVGSELSTTPLFDLSCKNSTTSSSSSVVSAAASSAAGSKAVGSSSGAQASATPSFTVGRPGVNGTVFGNGTYPLRPSGSASARPSAGAISSGSGSGSSGSGSSGSTGTSATSGQSSTSGSAAAGSSSPAAFSGASTLSGSLFGAVVAVFMTLAAL

SEQ ID NO: 22 - protein, 681 aa, Unknown
  Unknown
MAGVNRSFSYSRGDDALLRDDEREISPLRSAEDGLYSTSYGDISPLSAGFQGQTRPFDRGLVSVPEGQSLERHMTSTPGMDNLGPASVGGGISGIALGVANSNNRQSGVDAFRETDVPVRNLPAERDFNTTGSDNPYIPAPPDGDIYPNSETMRYRDSYSSHTGLGAGAPFAEHSTPGTTPSQRSFFDSPYQGVDAGPYQRHSAYSSHDYPLVINPDDIADDGDDGFPVHPKGVADYRSNGNVPAAGVAGAAAAGGLLGKFRALFKKEQPSPYYDSDIGGGLGGAEKAQGGRHIIGGGSRKRGWIVGLVLAAVIVAAIVGGAVGGILGHQEHDGDTSSSSSSSGTGSGGSDKGDGLLDKDSDEIKALMNNKNLHKVFPGVDYTPWGVQYPLCLQYPPSQNNVTRDLAVLTQLTNTIRLYGTDCNQTEMVLEAIDRLQLTNMKLWLGVWIDTNTTTTDRQISQLYKIVESANDTSIFKGAIVGNEALYRAGSDVASAETNLIGYINDVKDHFKEKNIDLPVGTSDLGDNWNAQLVSAADFVMSNIHPFFGGVEIDDAASWTWTFWQTHDTPLTAGTNKQQIISEVGWPTGGGNDCGSDNKCQNDKQGAVAGVDELNQFLSEWVCQALDNGTEYFWFEAFDEPWKVQYNTPGQEWEDKWGLMDSARNLKPGVKIPDCGGKTIT

SEQ ID NO: 23 - protein, 386 aa, Unknown
  Unknown
MKFSSSLLTLASLALANLSTALPKASPAPSSSSSSSSSASTSFASTSGLQFTIDGETGYFAGTNSYWIGFLTDDSDVDLVMSHLKSSGLKILRVWGFNDVTTQPSSGTVWYQLHQDGKSTINTGADGLQRLDYVVSSAEQHDIKLIINFVNYWTDYGGMSAYVSAYGGSDETDFYTSDTMQSAYQTYIKTVVERYSNSSAVFAWELANEPRCPSCDTSVLYDWIEKTSKFIKGLDADHMVCIGDEGFGLNTDSDGSYPYQFAEGLNFTKNLGIDTIDFGTLHLYPDSWGTSDDWGNGWISAHGAACKAAGKPCLLEEYGVTSNHCSVESPWQKTALNTTGVSADLFWQYGDDLSTGKSPDDGNTIYYGTSDYECLVTDHVAAIGSA

SEQ ID NO: 24 - protein, 1745 aa, Unknown
  Unknown
MRGKPPFVDNVPRRMHPSVEHIDTCVPVTALKALELRDVKLLLQAQGTYIRLIDEARGNLLAELKAFKRNHVHGFVALSQQEQAAGPSHARFIAWGGQSVRAFDLFLSVQEPSARLVASSAEYQGPDWILAGCASSQEESTTAYVLTAHNAVLGLHIVDGDGSKHEKAVHIKPLVTGVNTILYSADIVALSDSHILIAAGTVFGEIIVWSSYLNESGGAVGSIHHFFTGHEGSIFGVRISPSIASLRSDQSGRLLASCSDDRTIRIWDISDCERTSRHDAPAYSTDGFELRSTGFGAVAHDNEVGSEKTIASAFGHLARIWGVNFLPVGEGLGKVNLVSRGEDATCILWDLTWDPSSQTPQFKLTEGISIRKHTGKHVWSLEVRSTDTEAVIYTGGADGAVKNFTIKADENGSLVLPNLHDRITMTVDTQNPEPHVETSIKGFDFVSQNKFIAVTARGEVQVGHINAQDLSKQHIFKETLFVEDDLRSYSVVGSLPQEGIALVGNARGSIRLYNHNVKTLIRLVDVGQRPLILIPLDYNEVSESEANLVFTVSYPNSEIAELFKVSLSGDGPCVDRITINLPYGFGMASASLVCGKQYLALGSLTGNFALYKVANTESIEPVMPPSKLHGREGLSYITSFSSLYGEEEQLHPYFLTCGRSGTYGVHKLVISEGAEPSISLQTLHLASLAFNCEIQGAYIDKVSQDLMIYGFQPMDFVLWNESAQTEVARHKCNGGRRAWAFQPNNTKAWAGSLLWIQSGFSGMEIHPDASRTLRSGSHGREVKAMSATQQGGLGPLFATGSEDTNVRIFTPRDPQSENRWGAFKCLRLLREHHTGLQSVGWSTDGRFLFTSGGYEQFFVWRTHSVPRFGLGTTSDGECPKSDPNSDLRTTSFDVLEVEDEQAEGSFLICLTYSNSTIKIFHYTSSTEGGSFTLLANGTYMSNCLTQANFLRNGSSLSLITASTDGYFTLWDLTSVLEPFYTITSPLRMKQTIQGASITPATISCENRYQIHWNSIKSLELADLSNTLSLIVAAGDDNSMTVTLLDTSIENGAATCTIAVPDAHAACITTTKILTQHVNPSDGTARFAVASSGNDHQVKIWWVDIDTKMSGADRIQISKAAERYSSVADISSLDVLHDASGRIGTTTNGPNWIGYLTTTENASLVLNYNFAAGGATIDNALVPAYPGDLASQFRLFEDVYAQKPETAPWDAKDAVFGVWIGINDIGNAYYSTDAATYTPKLISRLESLVEEVYKNGGRKFLFLNVPPTSRSPLFLDQGEEVVKQHAEYLAVFNENLEGMVEKFNKEKGDVTTVLYDSWSFMTKILDDPTAYGFPNATCIDDDGTSCGSLTERSPCFDFIRPIGIDDICRCEDLQHFLFEYPLFSTFGRFNLNKRRRRCLAKLVTSVLDWDSWVIMKFQSTLLLAAAAGSALAVPHGPGHKKRASVFEWFGSNESGAEFGTNIPGVWGTDYIFPDPSAISTLIDKGMNFFRVQFMMERLLPDSMTGSYDEEYLANLTTVIKAVTDGGAHALVDPHNYGRYNGEIISSTSDFQTFWENLAGQYKDNDLVMFDTNNEYHDMDQDLVLNLNQAAINGIRAAGATSQYIFVEGNSWTGAWTWVDVNDNMKNLTDPEDKIVYEMHQYLDSDGSGTSETCVSETIGKERVTEATQWLKDNKKVGFIGEYAGGSNDVCRSAVSGMLEYMANNTDVWKGASWWAAGPWWGDYIFSMEPPDGTAYTGMLDILEAYL

SEQ ID NO: 25 - protein, 334 aa, Unknown
  Unknown
MKFSTVVCGLAAAGGALAAPAKERSIKKRASPFQWFGSNESGAEFGQNNIPGVEGTDYTFPNTTAIQVLIDQGMNIFRVPFLMERMVPNQMTGPVDSAYLQGYSQVINYITSHGASAVIDPHNYGRYYNNIISSPSDFQTFWNTIASNFADNDGVIFDTNNEYHDMDESLVVQLNQAAIDGIRAAGATSQYIFVEGNSWTGAWTWTQVNDAMANLTDPQNKIVYEMHQYLDSDGSGTSDQCVNATIGQDRVASATAWLKQNGKKAILGEFAGGANSVCESAVTGLLDHLADNTDVWTGAIWWAAGPWWADYIFSMEPPSGIAYEQVLPLLQPYL

SEQ ID NO: 26 - protein, 414 aa, Unknown
  Unknown
MDRILALVLLPLAAVTAQQIGTIPEVHPKLTTWKCTTAGGCVQQDTSVVLEYLSHPIHEVGNSDVSCVVSGGLNQSLCPNEEECSKNCVVEGANYTSSGVHTDGDALTLNQYVQNGDQVVAASPRVYLLASDDEDGNYSMLQLLNQELSFDVDVSKLVCGMNGALYLSEMDVSGGRNSLNPAGAQYGSGYCDAQCGVQPFINGTVNTGSLGACCNEMDIWEANALATAYTPHPCSVASIYPCSGDECGSNGVCDKPGCGYNPYALGDHDYYGYGKTVDTSKPFTVVTQFLTDDNTTTGTLTEIRRLYVQDGTVIQPSPSDSVSSLTDSFCSTADSYFEPLGGMKGMGEALGRGMVLVFSIWNDPGQFMNWLDSGNAGPCNSTEGNPATIQAEHPDTAVTFSNIRWGDIGSTFQS

SEQ ID NO: 27 - protein, 403 aa, Unknown
  Unknown
MVRLSPVLLASIAGSGLPLYAQAAGLNTAAKAVGLKYFGTATDNPELSDTAYETELNNTQDFGQLTPANSMKWDATEPQQNTFTFSGGDQIANLAKANGQMLRCHNLVWYNQLPSWVTGGSWTNETLLAAMKNHITNVVTHYKGQCYAWDVVNEALNDDGTYRSNVFYQYIGEAYIPIAFATAAAADPDAKLYYNDYNIEYPGVKATAAQNIVKLVQSYGARIDGVGLQSHFIVGQTPSTSAQQQNMAAFTALGVEVAITELDIRMQLPETSAQLTQQATDYQSTVQACVNTDSCVGITLWDWTDKYSWVPSTFSGWGDACPWDDNYQKKPAYNGILTALGGTPSSSTSYTLTPTTTSSGGSGSPTDVAQHWEQCGGLGWTGPTVCASGFTCTVINEYYSQCL

SEQ ID NO: 28 - protein, 261 aa, Unknown
  Unknown
MLVSPSFKMKPFIAVALSLPLAATLTTAAPTPTKTLQRRADFCGQWDSTVTGSYTVYNNLWGEGSASSGSQCTGVDSLDGNTLAWHTLWTWEGGSSSVKSFANAAYAFTATQLSQISSIPTTWQWSYTGTSIDADVAYDLFTSSSPSGSNEYEIMIWLAALGGSFPISSTGTTPIASPTIGGVSWNLYSGPNGATTVYSFVAATEQTDFSGDINDFLAYLQENQGLSSSQYLLSIQAGTEPFTGEDAELKTTAYSVSVLTS

SEQ ID NO: 29 - protein, 411 aa, Unknown
  Unknown
MKTVTTLSTLCALCGLATAWLPGIHKDITSIDGRNHFNTSSDNKRWLPASGKIRGVDLGSLFVTEPWMASNAWSSMGCGNAPSEFDCVMALGQDAANSAFKNHWSSWITKDDITEMQSYGLNTIRIPVGYWIKEDIVYSDSEHFPQGGLSYLEQVCGWASDAGFYIIIDLHGAPGAQVPKNADTGQYAPTAGFYVDYQYERALEFLEWMTTNIHTNNNFRNVGMLEIVNEPIQDANQVASMRTSYYPNAFKRIRAAEQKLGITQNNYIHIQMMNAKWGSGDPNEALTDTYFAAYDDHRYLKWDTSVPVSKDSYLSTSCNDDRGGNTPTIVGEFSLSPPDNVQWTSDWDPNSNKDFYQKWFAAQVMSYEKQNGWIFWSWKTDLGDYRWSYKQAVEAGVIPKGLDSVYNMGAC

SEQ ID NO: 30 - protein, 628 aa, Unknown
  Unknown
MQVSRIAALAALLQGAWAQAGPYAQCGGIGYSGSTVCAAGYTCTSQNPYYYQCVPATATTTTTTSSASASSTSSAPSTTCAGTFTPISAADFVANLNPGWNLGNTLDATPDEGSWNNPPVVSSTFDEVKAAGFKSVRLPVTYAYHFIGDSPDWTINATWLQRVSDVVDMITSRGLYTIVNAHHDSWIWADVTQPGANLTMIEEKFYRLWYQVGSKLACKSSLVAFEPINEPPCNDATDAAEINKLNTIFLKAINDAGGFNSQRVVTLVGGGEDSVKTSEWFVAPTGYSNPYAIQFHYYNPYDFIFSAWGKTIWGSDSDKSTLSTDLQLIRNNFTTVPLLIGEYDASPTNCETAARWKYFDYLIRTARALNISTIMWDNGQDHLDRTTGVWRDPSAVDIIMDATSGITNSLPDSTEDPSATTQWSSAYIFHKYGDPVSDQSLPFLFNGNSVSSISASDGTKLTPETDYVVAGSNITFKASFLSKYLSSTTAPGILANLTVSFSAGASEVIQLVQWTTPSLSSTSVAASAVNGSDLYIPITWGGIPKPAAVKAVEANGEHLVDSWTEYLPVIQQGRTTYSSQWNWDDSHIIITAATISTVLAAGQTTVFTFEFYPRDNGVVNAVNFTLTV

SEQ ID NO: 31 - protein, 254 aa, Unknown
  Unknown
MFTSQEDRESIKSDEKEAVPPIDLSAVAIVFVMNLKLFVSVSALLLTPLASALTGTTTTTWDCCKPACSWTQNAQAGGASGTVATCNINNQVLSDGATAQSACQGGNAYSCSDFQPIIISDTLSYGFAGNWETSNCCKCFQFTWTSGEGAGKSMIVQVVNSGGVNTGDFDIYTPGGGVGDYNACTSQYGAPPQGWGNQYGGVSSDAECDQLPSNLQPGCHWRFEWAGGGINGWTTNYEEVECPSQLTSISGCYP

SEQ ID NO: 32 - protein, 1506 aa, Unknown
  Unknown
MRYRDGEAVAFVRHDADVQQALDLTEPGLAPDAAVRPPPPRVLQSWSLIMNEQSGTFLFLASGFCRRHLLDGETMDRRLDFVRFFAPFITPRRGNALPAAFLWRTHSDRPDSDEGVSTILIRHPSILALIHDYSSMHVAHRWAVMSVDVLLPRRAGYLAWYTSLLPGLDLGYRPLQPASSSEDNLPPRTMAVTIRRFTRRSLLVLVSKTTILVTLVSLLLWLLVNTNIESAFDLLNLLPLPSPSPSPALAYTDGGYSLQRHSSQPPEAGSRSSSSASHNYTPPFHTAGRYILDAQNQRVKLASINWYGGSDEDFVPSGLDVQPRDRIAALIRDLGFNSVRLPYSDEMVRDNPLIPASRLAANRDLVDPDTGGASARDVFAAVVESLTDAGLLVIVNNHITQATWCCGANLCDAGWANDWFGGQWFCRVSQTTEEWIEHWETVMRPLAHNPRVIGADLRNEPRGLWGTLHWDDWVAAAERAAERLLALNPDWLIIVEGISSANDLSGVRTRPVRLPPPFAADRVVYSAHVYSWSGWGSLYPYSRRTYEDFVASMRGNWAYLLEEDLAPVWVGELGTPDQPTEGDCNYWTHLVEFLRVTDASWGYWALNPRKPADHEWESYGLTCNDWACVPVSHPVINWTRRRDEVHGATMTNSDSGPLAETSGSMLAPVACLEAAPPLPATAFSPSRPRSARPSVCLSVCLSVCLSVCLSVCRARARPRTDTAKSITHQKLRWKNPMLCSTDDGGYPAAWRWASHWRTSLSRTPRLARARTHDRSSGGAPHLANARGVCYRQFGEGFLPMTPRARAPSPPFSVPIGQSVLAADTDDITQGLKTPWFYGQRRREYTGSGGALRKVETGNGYNNRHPAHARGLQCEWPLGIAPALRPPLGRGHVGSCFPAQSPARRPPRPPNSARPSPQPPPSNEIAMMCSRRRLTGEESGRSPAALCPPGRVWVQTPRVAPSQPLIIAPCLSSAHVVHAQKLALAGSSADAAAGRPWLREDSAAIEPGAEDLHRVHAHRPRQCPDLRHAPVLGAVPPLEGDPGRVATTAVGQEHCQRGWERDTAVRRQSAGDADIALLAASDDVRRPGPTGGGGGWRGGACDHPAELLRGSRHAADHVERARQSSPGGRPVYLAMEQKETKAPEKAATLISMFQGQFRDICSTFHPAGLPGEIAGKSSNVAFAARHIIEAHRRDETVNPRDVIITVMDADTHLSQDYFTEIRRLHYRHIDEADRSFYASPIIFDRNSNEVPVFPHHDPHVGLFAAPGPRGEGWWVGWGSHGDWRGHAHAAQMLLLHGRGHHFAGDLHPGQPVQRLEQRRRGLAAFAGDLHGAVSPGPAAHVGSAGHGVCGAAEPGPVDRQGAAAHAPAAAAPGVVPSAVGGAFPAVPFHDPAAVLVDLHVCDAGVADPPDAGVDVLVHGGAAVRVVRVDEHLPDAVRSVARGVCQRARAGHGAGGTAGCGLLVPDVVAWEAPHRAGVLPDRGDDLRVDSVGACGDFAFLDGAAGVSG

SEQ ID NO: 33 - protein, 473 aa, Unknown
  Unknown
MAAGFLRVSGTKIVDANGTPVLLRGTALGGWMNMENFITGFPGHESTHRAAMLAVLGKEKYDYFFDKFLEYFFTEKDAQFCKSLGINCLRLPFNYRHFEDDMNPRVLKEEGFKHLDRVVDLCAKYQIYTILDMHTLPGGQSPGWHADNLTSHASFWDHRDHQDRTVWLWQQIAARYKSNPWIAGYNLINEPCDPQHVRLPAFYVRLEKAIHEIDPDHILFLDGNTFAAEWKGFDEYPILPNAVYSLHDYSRLGFPGPEQFTGSQEQLERLERQFLRKAEFHLSRNAPIWNGEFGPVYANPQYEEDADAINRQRYELLNAQLRLYDKYAIPWSIWLYKDIGLQGMLHTSPSSPWNKLLAPFLEKKKTLQLDAWGKYPSQEIDALLGPLVEWIDRVSPTAKSTYPSTWDTRRHIERAVLQTFLAESFQKEFAELFRDKSMKELDELARSFAFEQCVQRTELNKILSKHAEASGLA

SEQ ID NO: 34 - protein, 225 aa, Unknown
  Unknown
MLTKNLLLCFAAAKAALAVPHDSVAQRSDALHMLSERSTPSSTGENNGFYYSFWTDGGGDVTYTNGDAGAYTVEWSNVGNFVGGKGWNPGSAQDITYSGTFTPSGNGYLSVYGWTTDPLIEYYIVESYGDYNPGSGGTYKGTVTSDGSVYDIYTATRTNAASIQGTATFTQYWSVRQNKRVGGTVTTSNHFNAWAKLGMNLGTHNYQIVATEGYQSSGSSSITVQ

SEQ ID NO: 35 - protein, 231 aa, Unknown
  Unknown
MVAYSSLLLALSAASSAVALPNGKALLDMAKRSLTSSAEGESNGYFYSFWTNGEGDVTYTNGDAGEYTVEWTDCGDFVAGKGWNPGSAQAVTYSGSWETDANAYLSVYGWTTSPLVEFYIVDKYGDYDPSSGLTELGTVDSDDGTYKIYQTTREDADSIEGTATFKQYWSVRTEGRIGGTVTTQNHFDAWENLGLELGTFNYMIVATEGYESSGSATITVETSSDSTEESC

SEQ ID NO: 36 - protein, 256 aa, Unknown
  Unknown
MVSFLGQARLAVPILSAFACMLAASSAIPPPPRGALSPERLQWIREVIGNQTENDSVSDLAKRSTVLSTSQDGVDSAGFYYSVYNDNGADVGYTEYPTTGQFELGWSAEAEFLAGKGFKGGNPRSLTWDGYFTAEGDWTLAIYGWTTNPVTEWYIVETHGTGTPGNGDILGQVDSDGGVYDVYNLPYRNVPEIYGVTNFDQYWSVRRTHRTTGTVDVSAHFQGWKNLGLNPGSPVFQMVTLEGFSGQGYLDFTVSA

SEQ ID NO: 37 - protein, 342 aa, Unknown
  Unknown
MKTFGAASLITALLAASEGANAFTKTNTSPLKEVAESKGILIGSGAVNPNYLNDSLFATVLADQFQSLAPENELKWTFIHPTPNQYNWNATDRLVSFAEKHSMVVKGHGLISSCCNPDYLLNITDPKQFRAAMVTHFDAIMHRYAGKMDRWDVVIEALKTMGGGLQVNDFYKVLGPGYIADAFHIARAAGPEAKLFLSESLVETYPGKRQELYDLVSGLVSDNVPIDGVALQMHVTEAAPIPGVITDIVKSYNALGLEVSISEMDVHTLNTTLETDIYNAVLTEALGAGITDITFWGFTDKHAYTWIKGAKPLMFDEYYNPKGEFYATHTALTSFDNTTSPK

SEQ ID NO: 38 - protein, 311 aa, Unknown
  Unknown
MVQIKVAALAMLFASQVLSEPIEPRQASVSIDTKFKAHGKKYLGNIGDQYTLTKNSKTPAIIKADFGALTPENSMKWDATEPSRGQFSFSGSDYLVNFAQSNNKLIRGHTLVWHSQLPSWVQSITDKNTLIEVMKNHITTVMQHYKGKIYAWDVVNEIFNEDGSLRDSVFYKVIGEDYVRIAFETARAADPNAKLYINDYNLDSASYPKLTGMVSHVKKWIAAGIPIDGIALNALAGAGTKEIAVTELDIAGASSTDYVEVVEACLNQPKCIGITVWGVADPDSWRSSSTPLLFDSNYNPKPAYTAIANAL

SEQ ID NO: 39 - protein, 685 aa, Unknown
  Unknown
MAGVNRSFSYSRGDDALLRDDEREISPLRSAEDGLYSTSYGDVSPLSAGVQAQNRPFDRGLVSVPEGQTLERHMTSTPGMDNLGPASVGGGISGIALGVANSHNRQSGVDAFRETDVPVRNLPAERDFNTTGSDNPYIPAPPDGDIYPSSEAVRYRDSYSSHTGLGAGAPFAEHSTPGTTPSQRSFFDSPYQGVDAGPYQRHSAYSSHDYPLVINPDDIADDGDDGFPVHPKGAADYRSNANVPGTGVAGAAAAGGFLGKFRALFKREEPSPFYDSDIGGGLGGAEKAQGGRHIIGGGSRKRGWIVGLILAAVIVAAIVGGAVGGILGHQEHDGDTSSSSSSSSSSSGTGSGGSDKGDGLLDKDSDEIKALMNNKNLHKVFPGVDYTPWGVQYPLCLQYPPSQNNVTRDLAVLTQLTNTIRLYGTDCNQTEMVLEAIDRLQLTNMKLWLGVWIDTNTTTTDRQISQLYKIVENANDTSIFKGAIVGNEALYRAGSDVASAETNLIGYINDVKDHFKDKNIDLPVGTSDLGDNWNAQLVSAADFVMSNIHPFFGGVEIDDAASWTWTFWQTHDTPLTAGTNKQQIISEVGWPTGGGNDCGSDNKCQNDKQGAVAGIDELNQFLSEWVCQALDNGTEYFWFEAFDEPWKVQYNTPGQEWEDKWGLMDSARNLKPGVKIPDCGGKTIT

SEQ ID NO: 40 - protein, 739 aa, Unknown
  Unknown
MPTSTLLWSVGSLALSSMVLPAAASSYQLVETWKGEDFLTAFDFYTGADPTNGFVTYANQSYAESTGLVKVNSNGTFYMGVDHTTKLSTNGPGRESVRIGSNKYYDEGLFIIDLQHMPGSVCGTWPAFWSTGKNWPADGEIDIIEGVNKNEANEIVLHTSGTCQVSSQKMSGTLTSTECGEDAGTTGCVVEGTQGSSGTPFNENGGGVYAMQWTDEFLKFWFFPRGSIPSSITKGDPDVAAFGTPMAHMEGSCSIAEHFKAQQFIFDTTFCGDWAGGVYSTSGCPVSDSSSSFKSCVAYVAENPTAFAESYWEINYIKIYQTGVAASASASASHVESAASVAETISAVREGTNSVVATTAAATIAVTNTADAETATTMAEATTVAASTETSAADENGSSASTSTHYVTMTTTICPIAESSSAAAALAGGSSEATEASNSEGSPAAATPSSVTGASAEANESESTSAAVTTPSTATGASAEANGSESSSASEAGSVAGATPSSVSTTGASGEADSSEGASAAATPSNVSSTGASAEANGSEDSSASSEAKTVASATPSSVTGASAEANGNDSASSNAATASNVSGASAQAGDNESTPASAGANAGSSAAPSSVSGASAEANGSEGSSSHSSGSQAGAHSYGSVPSSAAAYGRPAPSSSSHAFATAPSSSGSSRVPTSAAAANNAAAATQGSSASGSNSGSSGHGSSSATTPSTPVFTGGASKLTLGASSVLSVLAFALLA

SEQ ID NO: 41 - protein, 427 aa, Unknown
  Unknown
MRRTATLLSALGLTAQLSSAAYTLQDDYSGSGFFDGFSFFTDTDPTNGFVDYVDEATAQSNGYISTSGDSVYMGVDHTNVAGSSGRQSVRISSDATYNHGLFILDLEHMPGGICGTWPAFWLVGADWPNNGEIDIIEGVNQQSGNDMTLHTSDGCSISSSSDFTGSMTTDNCYVYAAGQSSNAGCGITDPDATSYGTAFNANGGGVFATEWTSDAISIWFFERGSIPDDIDSGNPDPDSWGSPVARFQGDCDIDSHFDGLQIIFDTTFCGDWAGNVWGSGSCASVASSCSSYVANNPGAFVDAYWSINSLKVYQDDGDSTVAGVVDYGDDDDEDEDDDQDDGDDDSDDDDDDDDDSDSDDDSDDDGDDDDDDDDDDDDDEDSRPWRGGRNHHGQMLNASTSTSSFPSPSFVKKARWEPRNYMAGMIF

SEQ ID NO: 42 - protein, 383 aa, Unknown
  Unknown
MKLSNALLTLASLALANVSTALPKASPAPSTSSSAASTSFASTSGLQFTIDGETGYFAGTNSYWIGFLTDNADVDLVMGHLKSSGLKILRVWGFNDVTSQPSSGTVWYQLHQDGKSTINTGADGLQRLDYVVSSAEQHDIKLIINFVNYWTDYGGMSAYVSAYGGSGETDFYTSDTMQSAYQTYIKTVVERYSNSSAVFAWELANEPRCPSCDTSVLYNWIEKTSKFIKGLDADRMVCIGDEGFGLNIDSDGSYPYQFSEGLNFTMNLGIDTIDFGTLHLYPDSWGTSDDWGNGWITAHGAACKAAGKPCLLEEYGVTSNHCSVEGSWQKTALSTTGVGADLFWQYGDDLSTGKSPDDGNTIYYGTSDYQCLVTDHVAAIGSA

SEQ ID NO: 43 - protein, 335 aa, Unknown
  Unknown
MFAKLSLLSLLFSSAALGASNQTLSYGNIDKSATPEARALLKYIQLQYGSHYISGQQDIDSWNWVEKNIGVAPAILGSDFTYYSPSAVAHGGKSHAVEDVIQHAGRNGINALVWHWYAPTCLLDTAKEPWYKGFYTEATCFNVSEAVNDHGNGTNYKLLLRDIDAIAAQIKRLDQAKVPILFRPLHEPEGGWFWWGAQGPAPFKKLWDILYDRITRYHNLHNMVWVCNTADPAWYPGNDKCDIATIDHYPAVGDHGVAADQYKKLQTLTNNERVLAMAEVGPIPDPDKQASENVNWAYWMVWSGDFIEDGKQNPNQFLHKVYNDTRVVALNWEGA

SEQ ID NO: 44 - protein, 464 aa, Unknown
  Unknown
MLSKMQLAQLAAFAMTLATSEAAYQGFNYGNKFSDESSKFQADFEAEFKAAKNLVGTSGFTSARLYTMIQAYSTSDVIEAIPAAIAQDTSLLLGLWASGGGMDNEITALKTAISQYGEELGKLVVGISVGSEDLYRNSVEGAEADAGVGVNPDELVEYIKEVRSVIAGTALADVSIGHVDTWDSWTNSSNSAVVEAVDWLGFDGYPFFQSSMANSIDNAKTLFEESVAKTKAVAGDKEVWITETGWPVSGDSQGDAVASIANAKTFWDEVGCPLFGNVNTWWYILQDASPTTPNPSFGIVGSTLSTTPLFDLSCKNSTTSSSSAVVSAAASSAAGSKAVGSSQASSGAAAWATSASGSAKPTFTVGRPGVNGTVFGNGTYPLRPSGSASARPSAGAISSGSGSSSSGSGSSGSTGTSATSGQSSSSGSSAAAGSSSPAAFSGASTLSGSLFGAVVAVFMTLAAL

SEQ ID NO: 45 - protein, 410 aa, Unknown
  Unknown
MKTLSLAAVLLVQAWTANSSPRAKRSSGFQWFGSNESGAEFGSGNIPGTLGTDYIWPDATAIATLHSAGMNIFRVPFLMERLVPDELTGAADATYMADLKATVQTITDLGAYAVVDPHNFGRYYGNIITSTSDFAAFWTTVASEFTDNDLVIFDTNNEFHDEDQTLVLDLNQAAITAIRATGATTQYIFVEGNSYTGAWTWTTTNTNLVNLTDPNDHLIYEMHQYLDSDGSGTSSTCVSSTIGAERIADATTWLKENGKQAVLGEFAGGANSVCEEAVTGMLDAMVDASDVWLGGMWWSAGPWWGDYIFSLEPDDGIAYEYYLGVLEGYTPGSSSGSSGGSTTSAVASASSTSSAGSTTSKVTTTTAATATSTAVAAHYAQCGGEGWTGATTCADGYTCTVENEWYSQCL

SEQ ID NO: 46 - protein, 241 aa, Unknown
  Unknown
MKVLALSALLSLASAASISRRSDFCGQWDTATAGDFILYNDLWGEDNASSGSQCTGVDSASGSEIAWHTSWSWEGGSSDVKSYANAALQFTGTQLSSISSIPSTWKWTYSGSDIVADVAYDMFLGSTADASSDEYEIMVWLAALGGAGPISSTGSTIATPTINGVTWDLYTGPNGDTTVYSFVAQSTTEDFSGDLNDFFTYLVDNEGVSDSLYLTTLEAGTEPFTGSDAELKVSEYSVSIE

SEQ ID NO: 47 - protein, 248 aa, Unknown
  Unknown
MNRYLSIPLCLASAVPALAGLAARDPIGTICTKNNIITTDDFILYNNLWGEDYATSGSECTYLDYDSGNSISWQTSWTWAGGDDYVKSYPNAVLNVGAKQLSTITSIPSTWKWSYTGNDLVADVSYDAFLSTTDSTTATHEYEIMIWLAAYGGIEPIGNSDGPIASPTIGGYTWDLYKGPNDWTVYSFVARETITDFSADVLEFFTYLVDNEGVSSSLYLQTLGAGTEPKTGSDAWFTVSPYTVSINT

SEQ ID NO: 48 - protein, 517 aa, Unknown
  Unknown
MRISNLIVAASAASMVSALPSRQMKKRDSGFKWVGTSESGAEFGSALPGTLGTDYTWPETSKIQVLRNKGMNIFRIPFLMERLTPDGLTSSFASTYLSDLKSTVEFVTNSGAYAVLDPHNYGRFDGSIITSTSDFKTWWKNVATEFADNDKVIFDTNNEYHDMEQSLVLDLNQAAINGIRAAGATTQYIFVEGNAYTGAWDWTTYNDNLSGLTDSEDKIIYEMHQYLDSDSSGTSETCVSSTIGQERLEKATEWLKTNNKQGIVGEFAGGVNSVCEEAVEGMLAYMSENSDVWVGASWWSAGPWWGTYMYSLEPTDGTAYSTYLPILEKYFPSGDASASSSASVSVAAATSTASTTTAAFEQTTTPATQVEIASSSSSSSANAASQTTLSKVKSKSKSPCKLSSATSSAVAATTPVVVATTPAVAPTSSSVAFVTTSVYVPTTTAAVAPSQVSSSAAASSSGVVGVSDPQGPSATNSAGEVNQYYQCGGINWTGPTVCASPYTCKVQNDYYYQCVAE

SEQ ID NO: 49 - protein, 331 aa, Unknown
  Unknown
MKFQSTLLLAAAAGSALAVPHGSGHKKRASVFEWFGSNESGAEFGTNIPGVWGTDYIFPDPSTISTLIGKGMNFFRVQFMMERLLPDSMTGSYDEEYLANLTTVVKAVTDGGAHALIDPHNYGRYNGEIISSTSDFQTFWQNLAGQYKDNDLVMFDTNNEYYDMDQDLVLNLNQAAINGIRAAGASQYIFVEGNSWTGAWTWVDVNDNMKNLTDPEDKIVYEMHQYLDSDGSGTSETCVSGTIGKERITDATQWLKDNKKVGFIGEYAGGSNDVCRSAVSGMLEYMANNTDVWKGASWWAAGPWWGDYIFSLEPPDGTAYTGMLDILETYL